European Patent Specification EP 3 418 299 B1, published November 13, 2024. Title: HOMOGENEOUS ANTIBODY POPULATIONS. Applicant: AMGEN INC. Application not yet assigned. The sequence listing filed with the application follows.

SEQUENCE LISTING (86 sequences)

SEQ ID NO: 1 - protein, 15 aa, human
EPKSCDKTHTCPPCP

SEQ ID NO: 2 - protein, 12 aa, human
ERKCCVECPPCP

SEQ ID NO: 3 - protein, 61 aa, human
ELKTPLDTTHTCPRCPEPKSCDTPPPCPRCPEPKSCDTPPPCPRCPEPKSCDTPPPCPRCP

SEQ ID NO: 4 - protein, 12 aa, human
ESKYGPPCPSCP

SEQ ID NO: 5 - protein, 17 aa, human
KCCVECPPCPAPPVAGP

SEQ ID NO: 6 - protein, 21 aa, human
KSCDKTHTCPPCPAPELLGGP

SEQ ID NO: 7 - protein, 10 aa, human
KCCVECPPCP

SEQ ID NO: 8 - protein, 10 aa, human
KSCVECPPCP

SEQ ID NO: 9 - protein, 10 aa, human
KCSVECPPCP

SEQ ID NO: 10 - protein, 10 aa, human
KSSVECPPCP

SEQ ID NO: 11 - protein, 26 aa, human
CCVECPPCPAPPVAGPSVFLFPPKPK

SEQ ID NO: 12 - protein, 12 aa, human
GPSVFPLAPCSR

SEQ ID NO: 13 - protein, 10 aa, human
RKCCVECPPC

SEQ ID NO: 14 - protein, 11 aa, human
  VARIANT 4: Xaa = Any Amino Acid
  VARIANT 4: Xaa = Any Amino Acid
RKCXCVECPPC

SEQ ID NO: 15 - protein, 12 aa, human
  VARIANT 4, 5: Xaa = Any Amino Acid
  VARIANT 4, 5: Xaa = Any Amino Acid
RKCXXCVECPPC

SEQ ID NO: 16 - protein, 13 aa, human
  VARIANT 4, 5, 6: Xaa = Any Amino Acid
  VARIANT 4, 5, 6: Xaa = Any Amino Acid
RKCXXXCVECPPC

SEQ ID NO: 17 - protein, 12 aa, human
  VARIANT 3, 5: Xaa = Any Amino Acid
  VARIANT 3, 5: Xaa = Any Amino Acid
RKXCXCVECPPC

SEQ ID NO: 18 - protein, 13 aa, human
  VARIANT 3, 5, 6: Xaa = Any Amino Acid
  VARIANT 3, 5, 6: Xaa = Any Amino Acid
RKXCXXCVECPPC

SEQ ID NO: 19 - protein, 13 aa, human
  VARIANT 3, 4, 6: Xaa = Any Amino Acid
  VARIANT 3, 4, 6: Xaa = Any Amino Acid
RKXXCXCVECPPC

SEQ ID NO: 20 - protein, 14 aa, human
  VARIANT 3, 4, 6, 7: Xaa = Any Amino Acid
  VARIANT 3, 4, 6, 7: Xaa = Any Amino Acid
RKXXCXXCVECPPC

SEQ ID NO: 21 - protein, 11 aa, human
  VARIANT 3: Xaa = Any Amino Acid
  VARIANT 3: Xaa = Any Amino Acid
RKXCCVECPPC

SEQ ID NO: 22 - protein, 12 aa, human
  VARIANT 3, 4: Xaa = Any Amino Acid
  VARIANT 3, 4: Xaa = Any Amino Acid
RKXXCCVECPPC

SEQ ID NO: 23 - protein, 4 aa, human
  VARIANT 4: Xaa = Any Amino Acid
  VARIANT 4: Xaa = Any Amino Acid
GECX

SEQ ID NO: 24 - protein, 5 aa, human
  VARIANT 4, 5: Xaa = Any Amino Acid
  VARIANT 4, 5: Xaa = Any Amino Acid
GECXX

SEQ ID NO: 25 - protein, 6 aa, human
  VARIANT 4, 5, 6: Xaa = Any Amino Acid
  VARIANT 4, 5, 6: Xaa = Any Amino Acid
GECXXX

SEQ ID NO: 26 - protein, 5 aa, human
  VARIANT 4: Xaa = Any Amino Acid
  VARIANT 4: Xaa = Any Amino Acid
GECXS

SEQ ID NO: 27 - protein, 6 aa, human
  VARIANT 4, 5: Xaa = Any Amino Acid
  VARIANT 4, 5: Xaa = Any Amino Acid
GECXXS

SEQ ID NO: 28 - protein, 7 aa, human
  VARIANT 4, 5, 6: Xaa = Any Amino Acid
  VARIANT 4, 5, 6: Xaa = Any Amino Acid
GECXXXS

SEQ ID NO: 29 - protein, 5 aa, human
  VARIANT 5: Xaa = Any Amino Acid
  VARIANT 5: Xaa = Any Amino Acid
GECSX

SEQ ID NO: 30 - protein, 6 aa, human
  VARIANT 5, 6: Xaa = Any Amino Acid
  VARIANT 5, 6: Xaa = Any Amino Acid
GECSXX

SEQ ID NO: 31 - protein, 7 aa, human
  VARIANT 5, 6, 7: Xaa = Any Amino Acid
  VARIANT 5, 6, 7: Xaa = Any Amino Acid
GECSXXX

SEQ ID NO: 32 - protein, 9 aa, human
CACVECPPC

SEQ ID NO: 33 - protein, 10 aa, human
CPPCVECPPC

SEQ ID NO: 34 - protein, 98 aa, human
VSGGSINSGDYYWSWIRQHPGKGLDCIGYIYYSGSTYYNPSLKSRVTISVDTSKNQFFLKLTSVTAADTAVYYCARSTVVNPGWFDPWGQGTLVTVSS

SEQ ID NO: 35 - protein, 105 aa, human
TITCQASQDINNYLNWFQQKPGKAPKVLIHDASNLETGGPSRFSGSGSGTDFTFTISGLQPEDIATYYCQQYESLPLTFGGGTKVEIKRTVAAPSVFIFPPSDEQ

SEQ ID NO: 36 - protein, 97 aa, human
VSGGSINSGDYYWSWIRQHPGKGLEWIGSIYYSGNTFYNPSLKSRVTISLDTSKNQFSLKLSSVTAADTAVCYCARNIVTTGAFDIWGQGTMVTVSS

SEQ ID NO: 37 - protein, 105 aa, human
TITCQASQDITIYLNWYQQKPGKAPKLLINDASSLETGVPLRFSGSGSGTDFTFTISSLQPEDIATYYCQQYDHLPLTFGGGTKVAIKRTVAAPSVFIFPPSDEQ

SEQ ID NO: 38 - protein, 96 aa, human
VSGGSISSGDYYWTWIRQHPGKGLEWIGYIYYSGNTYYNPSLKSRVSMSIDTSENQFSLKLSSVTAADTAVYYCARKPVTGGEDYWGQGTLVTVSS

SEQ ID NO: 39 - protein, 105 aa, human
TITCQASQDISNYLNWYQQKPGKAPKLLIYDASNLETGVPSRFSGSGSGTDFTFTISSLQPEDIVGYYVQQYESLPCGFGQGTKLEIKRTVAAPSVFIFPPSDEQ

SEQ ID NO: 40 - protein, 97 aa, human
VSGGSINSGDFYWSWIRQHPGKGLEWIGYIYYSGSTYYNPSLKSRVTMSIDPSKNQFSLKLISVTAADTAVYYCATSLYYGGGMDVWGQGTTVTVSS

SEQ ID NO: 41 - protein, 105 aa, human
  VARIANT 87: Xaa = Any Amino Acid
TITCQASQDISNNLNWYQQKRGNAPKLLIYDASNLETGVPSRFSGSGSGTDFTFTISNLQPEDIATYYCQHYDHLPWTFGQGTKVEXKRTVAAPSVFIFPPSDEQ

SEQ ID NO: 42 - protein, 97 aa, human
VSGGSINNGDYYWSWIRQHPGKGLEWIGHIYYSGSTYYIPSLKSRTTISVDTSKNQFSLKLNSVTAADTAVYYCARGTVTTYYFDYWGQGTTVTVSS

SEQ ID NO: 43 - protein, 107 aa, human
TITCRASQSISSYLNWYQQKPGKAPKLLIYAASSLQSGVPSRFSGSGSGTDFTLTISSLQPEDFATYYCQQGYRTPPECSFGQGTKLEIKRTVAAPSVFIFPPSDEQ

SEQ ID NO: 44 - protein, 97 aa, human
VSGGSVSSGDYYWSWIRQPPGKGLEWIGHLYYSGNTNYNPSLKSRVTISLDTSKNQFSLKLSSVTAADTAVYYCARDFLTGSFFDYWGQGTLVTVSS

SEQ ID NO: 45 - protein, 105 aa, human
TITCQASQDISNYLNWYQQKPGKAPKLLINDASDLETGVPSRISGSGSGTDFTFTISNLQPEDIATYYCQQYDSLPLTFGGGTKVEIRRTVAAPSVFIFPPSDEQ

SEQ ID NO: 46 - protein, 96 aa, human
VSGGSVYSGDYYWSWIRQPPGKGLEWIGYIYYSGSTNYNPSLKSRVTISVDTSKNQFSLKLSSVTAADTAVYYCARDSILGATNYWGQGTLVTVSS

SEQ ID NO: 47 - protein, 105 aa, human
  VARIANT 9, 15, 27, 51, 52, 70, 73: Xaa = Any Amino Acid
TITCQASQXISNYLXWYQQKPGKAPKXLISDASNLETGVPSRFSGSGSGTXXTFTISSLQPEDIATYHCXQYXSLPLTFGGGTKVEIKRTVAAPSVFIFPPSDEQ

SEQ ID NO: 48 - protein, 95 aa, human
VSGGSVSSGDYYWTWIRQSPGKGLEWIGHIYYSGNTNYNPSLKSRLTISIDTSKTQFSLKLSSVTAADTAIYYCVRDRVTGAFDIWGQGTMVTSS

SEQ ID NO: 49 - protein, 105 aa, human
TITCQASQDISNYLNWYQQKPGKAPKLLIYDASNLETGVPSRFSGSGSGTDFTFTISSLQPEDIATYFCQHFDHLPLAFGGGTKVEIKRTVAAPSVFIFPPSDEQ

SEQ ID NO: 50 - protein, 119 aa, human
VSGGSINSGDYYWSWIRQHPGKGLDCIGYIYYSGSTYYNPSLKSRVTISVDTSKNQFFLKLTSVTAADTAVYYCARSTVVNPGWFDPWGQGTLVTVSSASTKGPSVFPPLAPCSRSTST

SEQ ID NO: 51 - protein, 118 aa, human
VSGGSINSGDYYWSWIRQHPGKGLEWIGSIYYSGNTFYNPSLKSRVTISLDTSKNQFSLKLSSVTAADTAVCYCARNIVTTGAFDIWGQGTMVTVSSASTKGPSVFPPLAPCSRSTST

SEQ ID NO: 52 - protein, 117 aa, human
VSGGSISSGDYYWTWIRQHPGKGLEWIGYIYYSGNTYYNPSLKSRVSMSIDTSENQFSLKLSSVTAADTAVYYCARKPVTGGEDYWGQGTLVTVSSASTKGPSVFPPLAPCSRSTST

SEQ ID NO: 53 - protein, 118 aa, human
VSGGSINSGDFYWSWIRQHPGKGLEWIGYIYYSGSTYYNPSLKSRVTMSIDPSKNQFSLKLISVTAADTAVYYCATSLYYGGGMDVWGQGTTVTVSSASTKGPSVFPPLAPCSRSTST

SEQ ID NO: 54 - protein, 118 aa, human
VSGGSINNGDYYWSWIRQHPGKGLEWIGHIYYSGSTYYIPSLKSRTTISVDTSKNQFSLKLNSVTAADTAVYYCARGTVTTYYFDYWGQGTTVTVSSASTKGPSVFPPLAPCSRSTST

SEQ ID NO: 55 - protein, 118 aa, human
VSGGSVSSGDYYWSWIRQPPGKGLEWIGHLYYSGNTNYNPSLKSRVTISLDTSKNQFSLKLSSVTAADTAVYYCARDFLTGSFFDYWGQGTLVTVSSASTKGPSVFPPLAPCSRSTST

SEQ ID NO: 56 - protein, 117 aa, human
VSGGSVYSGDYYWSWIRQPPGKGLEWIGYIYYSGSTNYNPSLKSRVTISVDTSKNQFSLKLSSVTAADTAVYYCARDSILGATNYWGQGTLVTVSSASTKGPSVFPPLAPCSRSTST

SEQ ID NO: 57 - protein, 116 aa, human
VSGGSVSSGDYYWTWIRQSPGKGLEWIGHIYYSGNTNYNPSLKSRLTISIDTSKTQFSLKLSSVTAADTAIYYCVRDRVTGAFDIWGQGTMVTSSASTKGPSVFPPLAPCSRSTST

SEQ ID NO: 58 - protein, 467 aa, Mus musculus
MEFGLSWLFLVAILKGVQCEVQLLESGGGLVQPGGSLRLSCAASGFTFSSYAMSWVRQAPGKGLEWVSGITGSGGSTYAADSVKGRFTISRDNSKNTLYLQMNSLRAEDTAVYYCAKDPGTTVIMSWFDPWGQGTLVTVSSASTKGPSVFPLAPCSRSTSESTAALGCLVKDYFPEPVTVSWNSGALTSGVHTFPAVLPSSGLYSLSSVVTVPSSNFGTQTYTCNVDHKPSNTKVDKTVERKCCVECPPCPAPPVAGPSVFLFPPKPKDTLMISRTPEVTCVVVDVSHEDPEVQFNWYVDGVEVHNAKTKPREEQFNSTFRVVSVLTVVHQDWLNGKEYKCKVSNKGLPAPIEKTISKTKGQPREPQVYTLPPSREEMTKNQVSLTCLVKGFYPSDIAVEWESNGQPENNYKTTPPMLDSDGSFFLYSKLTVDKSRWQQGNVFSCSVMHEALHNHYTQKSLSLSPGK

SEQ ID NO: 59 - protein, 235 aa, Mus musculus
METPAQLLFLLLLWLPDTTGEIVLTQSPGTLSLSPGERATLSCRASQSVRGRYLAWYQQKPGQAPRLLIYGASSRATGIPDRFSGSGSGTDFTLTISRLEPEDFAVFRCQQYGSSPRTFGQGTKVEIKRTVAAPSVFIFPPSDEQLKSGTASVVCLLNNFYPREAKVQWKVDNALQSGNSQESVTEQDSKDSTYSLSSTLTLSKADYEKHKVYACEVTHQGLSSPVTKSFNRGEC

SEQ ID NO: 60 - protein, 122 aa, Mus musculus
EVQLLESGGGLVQPGGSLRLSCAASGFTFSSYAMSWVRQAPGKGLEWVSGITGSGGSTYYADSVKGRFTISRDNSKNTLYLQMNSLRAEDTAVYYCAKDPGTTVIMSWFDPWGQGTLVTVSS

SEQ ID NO: 61 - protein, 108 aa, Mus musculus
EIVLTQSPGTLSLSPGERATLSCRASQSVRGRYLAWYQQKPGQAPRLLIYGASSRATGIPDRFSGSGSGTDFTLTISRLEPEDFAVFYCQQYGSSPRTFGQGTKVEIK

SEQ ID NO: 62 - protein, 139 aa, human
MEFGLSWVFLVALLRGVQCQVQLVESGGGVVQPGRSLRLSCAASGFTFSNYGMHWVRQAPGKGLEWVAGIWNDGINKYHAHSVRGRFTISRDNSKNTLYLQMNSPRAEDTAVYYCARARSFDWLLFEFWGQGTLVTVSS

SEQ ID NO: 63 - protein, 128 aa, human
MEAPAQLLFLLLLWLPDTTGEIVLTQSPATLSLSPGERATLSCRASQSVSSYLAWYQQKPGQAPRLLIYDASNRATGIPARFSGSGSGTDFTLTISSLEPEDFAVYYCQQRSNWPPLTFGGGTKVEIK

SEQ ID NO: 64 - protein, 139 aa, human
MEFGLSWVFLVALLRGVQCQVQLVESGGGVVQPGRSLRLSCAVSGFTFSNYGMHWVRQAPGKGLEWVAAIWNDGENKHHAGSVRGRFTISRDNSKNTLYLQMNSLRAEDTAVYYCARGRYFDWLLFEYWGQGTLVTVSS

SEQ ID NO: 65 - protein, 137 aa, human
MGSTAILALLLAVLQGVCAEVQLMQSGAEVKKPGESLKISCKGSGYSFSFHWIAWVRQMPGKGLEWMGIIHPGASDTRYSPSFQGQVTISADNSNSATYLQWSSLKASDTAMYFCARQRELDYFDYWGQGTLVTVSS

SEQ ID NO: 66 - protein, 126 aa, human
MSPSQLIGFLLLWVPASRGEIVLTQSPDFQSVTPKEKVTITCRASQSIGSSLHWYQQKPDQSPKLLIKYASQSFSGVPSRFSGSGSGTDFTLTINSLEAEDAAAYYCHQSSSLPLTFGGGTKVEIK

SEQ ID NO: 67 - protein, 469 aa, human
MEFGLSWVFLVALLRGVQCQVQLVESGGGVVQPGRSLRLSCAASGFTFSNYGMHWVRQAPGKGLEWVAGIWNDGINKYHAHSVRGRFTISRDNSKNTLYLQMNSPRAEDTAVYYCARARSFDWLLFEFWGQGTLVTVSSASTKGPSVFPLAPSSKSTSGGTAALGCLVKDYFPEPVTVSWNSGALTSGVHTFPAVLQSSGLYSLSSVVTVPSSSLGTQTYICNVNHKPSNTKVDKKVEPKSCDKTHTCPPCPAPELLGGPSVFLFPPKPKDTLMISRTPEVTCVVVDVSHEDPEVKFNWYVDGVEVHNAKTKPREEQYNSTYRVVSVLTVLHQDWLNGKEYKCKVSNKALPAPIEKTISKAKGQPREPQVYTLPPSRDELTKNQVSLTCLVKGFYPSDIAVEWESNGQPENNYKTTPPVLDSDGSFFLYSKLTVDKSRWQQGNVFSCSVMHEALHNHYTQKSLSLSPGK

SEQ ID NO: 68 - protein, 465 aa, human
MEFGLSWVFLVALLRGVQCQVQLVESGGGVVQPGRSLRLSCAASGFTFSNYGMHWVRQAPGKGLEWVAGIWNDGINKYHAHSVRGRFTISRDNSKNTLYLQMNSPRAEDTAVYYCARARSFDWLLFEFWGQGTLVTVSSASTKGPSVFPLAPCSRSTSESTAALGCLVKDYFPEPVTVSWNSGALTSGVHTFPAVLQSSGLYSLSSVVTVPSSNFGTQTYTCNVDHKPSNTKVDKTVERKCCVECPPCPAPPVAGPSVFLFPPKPKDTLMISRTPEVTCVVVDVSHEDPEVQFNWYVDGVEVHNAKTKPREEQFNSTFRVVSVLTVVHQDWLNGKEYKCKVSNKGLPAPIEKTISKTKGQPREPQVYTLPPSREEMTKNQVSLTCLVKGFYPSDIAVEWESNGQPENNYKTTPPMLDSDGSFFLYSKLTVDKSRWQQGNVFSCSVMHEALHNHYTQKSLSLSPGK

SEQ ID NO: 69 - protein, 466 aa, human
MEFGLSWVFLVALLRGVQCQVQLVESGGGVVQPGRSLRLSCAASGFTFSNYGMHWVRQAPGKGLEWVAGIWNDGINKYHAHSVRGRFTISRDNSKNTLYLQMNSPRAEDTAVYYCARARSFDWLLFEFWGQGTLVTVSSASTKGPSVFPLAPCSRSTSESTAALGCLVKDYFPEPVTVSWNSGALTSGVHTFPAVLQSSGLYSLSSVVTVPSSSLGTKTYTCNVDHKPSNTKVDKRVESKYGPPCPSCPAPEFEGGPSVFLFPPKPKDTLMISRTPEVTCVVVDVSQEDPEVQFNWYVDGVEVHNAKTKPREEQFNSTYRVVSVLTVLHQDWLNGKEYKCKVSNKGLPSSIEKTISKAKGQPREPQVYTLPPSQEEMTKNQVSLTCLVKGFYPSDIAVEWESNGQPENNYKTTPPVLDSDGSFFLYSRLTVDKSRWQEGNVFSCSVMHEALHNHYTQKSLSLSLGK

SEQ ID NO: 70 - protein, 469 aa, human
MEFGLSWVFLVALLRGVQCQVQLVESGGGVVQPGRSLRLSCAVSGFTFSNYGMHWVRQAPGKGLEWVAAIWNDGENKHHAGSVRGRFTISRDNSKNTLYLQMNSLRAEDTAVYYCARGRYFDWLLFEYWGQGTLVTVSSASTKGPSVFPLAPSSKSTSGGTAALGCLVKDYFPEPVTVSWNSGALTSGVHTFPAVLQSSGLYSLSSVVTVPSSSLGTQTYICNVNHKPSNTKVDKKVEPKSCDKTHTCPPCPAPELLGGPSVFLFPPKPKDTLMISRTPEVTCVVVDVSHEDPEVKFNWYVDGVEVHNAKTKPREEQYNSTYRVVSVLTVLHQDWLNGKEYKCKVSNKALPAPIEKTISKAKGQPREPQVYTLPPSRDELTKNQVSLTCLVKGFYPSDIAVEWESNGQPENNYKTTPPVLDSDGSFFLYSKLTVDKSRWQQGNVFSCSVMHEALHNHYTQKSLSLSPGK

SEQ ID NO: 71 - protein, 465 aa, human
MEFGLSWVFLVALLRGVQCQVQLVESGGGVVQPGRSLRLSCAVSGFTFSNYGMHWVRQAPGKGLEWVAAIWNDGENKHHAGSVRGRFTISRDNSKNTLYLQMNSLRAEDTAVYYCARGRYFDWLLFEYWGQGTLVTVSSASTKGPSVFPLAPCSRSTSESTAALGCLVKDYFPEPVTVSWNSGALTSGVHTFPAVLQSSGLYSLSSVVTVPSSNFGTQTYTCNVDHKPSNTKVDKTVERKCCVECPPCPAPPVAGPSVFLFPPKPKDTLMISRTPEVTCVVVDVSHEDPEVQFNWYVDGVEVHNAKTKPREEQFNSTFRVVSVLTVVHQDWLNGKEYKCKVSNKGLPAPIEKTISKTKGQPREPQVYTLPPSREEMTKNQVSLTCLVKGFYPSDIAVEWESNGQPENNYKTTPPMLDSDGSFFLYSKLTVDKSRWQQGNVFSCSVMHEALHNHYTQKSLSLSPGK

SEQ ID NO: 72 - protein, 466 aa, human
MEFGLSWVFLVALLRGVQCQVQLVESGGGVVQPGRSLRLSCAVSGFTFSNYGMHWVRQAPGKGLEWVAAIWNDGENKHHAGSVRGRFTISRDNSKNTLYLQMNSLRAEDTAVYYCARGRYFDWLLFEYWGQGTLVTVSSASTKGPSVFPLAPCSRSTSESTAALGCLVKDYFPEPVTVSWNSGALTSGVHTFPAVLQSSGLYSLSSVVTVPSSSLGTKTYTCNVDHKPSNTKVDKRVESKYGPPCPSCPAPEFEGGPSVFLFPPKPKDTLMISRTPEVTCVVVDVSQEDPEVQFNWYVDGVEVHNAKTKPREEQFNSTYRVVSVLTVLHQDWLNGKEYKCKVSNKGLPSSIEKTISKAKGQPREPQVYTLPPSQEEMTKNQVSLTCLVKGFYPSDIAVEWESNGQPENNYKTTPPVLDSDGSFFLYSRLTVDKSRWQEGNVFSCSVMHEALHNHYTQKSLSLSLGK

SEQ ID NO: 73 - protein, 467 aa, human
MGSTAILALLLAVLQGVCAEVQLMQSGAEVKKPGESLKISCKGSGYSFSFHWIAWVRQMPGKGLEWMGIIHPGASDTRYSPSFQGQVTISADNSNSATYLQWSSLKASDTAMYFCARQRELDYFDYWGQGTLVTVSSASTKGPSVFPLAPSSKSTSGGTAALGCLVKDYFPEPVTVSWNSGALTSGVHTFPAVLQSSGLYSLSSVVTVPSSSLGTQTYICNVNHKPSNTKVDKKVEPKSCDKTHTCPPCPAPELLGGPSVFLFPPKPKDTLMISRTPEVTCVVVDVSHEDPEVKFNWYVDGVEVHNAKTKPREEQYNSTYRVVSVLTVLHQDWLNGKEYKCKVSNKALPAPIEKTISKAKGQPREPQVYTLPPSRDELTKNQVSLTCLVKGFYPSDIAVEWESNGQPENNYKTTPPVLDSDGSFFLYSKLTVDKSRWQQGNVFSCSVMHEALHNHYTQKSLSLSPGK

SEQ ID NO: 74 - protein, 463 aa, human
MGSTAILALLLAVLQGVCAEVQLMQSGAEVKKPGESLKISCKGSGYSFSFHWIAWVRQMPGKGLEWMGIIHPGASDTRYSPSFQGQVTISADNSNSATYLQWSSLKASDTAMYFCARQRELDYFDYWGQGTLVTVSSASTKGPSVFPLAPCSRSTSESTAALGCLVKDYFPEPVTVSWNSGALTSGVHTFPAVLQSSGLYSLSSVVTVPSSNFGTQTYTCNVDHKPSNTKVDKTVERKCCVECPPCPAPPVAGPSVFLFPPKPKDTLMISRTPEVTCVVVDVSHEDPEVQFNWYVDGVEVHNAKTKPREEQFNSTFRVVSVLTVVHQDWLNGKEYKCKVSNKGLPAPIEKTISKTKGQPREPQVYTLPPSREEMTKNQVSLTCLVKGFYPSDIAVEWESNGQPENNYKTTPPMLDSDGSFFLYSKLTVDKSRWQQGNVFSCSVMHEALHNHYTQKSLSLSPGK

SEQ ID NO: 75 - protein, 464 aa, human
MGSTAILALLLAVLQGVCAEVQLMQSGAEVKKPGESLKISCKGSGYSFSFHWIAWVRQMPGKGLEWMGIIHPGASDTRYSPSFQGQVTISADNSNSATYLQWSSLKASDTAMYFCARQRELDYFDYWGQGTLVTVSSASTKGPSVFPLAPCSRSTSESTAALGCLVKDYFPEPVTVSWNSGALTSGVHTFPAVLQSSGLYSLSSVVTVPSSSLGTKTYTCNVDHKPSNTKVDKRVESKYGPPCPSCPAPEFEGGPSVFLFPPKPKDTLMISRTPEVTCVVVDVSQEDPEVQFNWYVDGVEVHNAKTKPREEQFNSTYRVVSVLTVLHQDWLNGKEYKCKVSNKGLPSSIEKTISKAKGQPREPQVYTLPPSQEEMTKNQVSLTCLVKGFYPSDIAVEWESNGQPENNYKTTPPVLDSDGSFFLYSRLTVDKSRWQEGNVFSCSVMHEALHNHYTQKSLSLSLGK

SEQ ID NO: 76 - protein, 235 aa, human
MEAPAQLLFLLLLWLPDTTGEIVLTQSPATLSLSPGERATLSCRASQSVSSYLAWYQQKPGQAPRLLIYDASNRATGIPARFSGSGSGTDFTLTISSLEPEDFAVYYCQQRSNWPPLTFGGGTKVEIKRTVAAPSVFIFPPSDEQLKSGTASVVCLLNNFYPREAKVQWKVDNALQSGNSQESVTEQDSKDSTYSLSSTLTLSKADYEKHKVYACEVTHQGLSSPVTKSFNRGEC

SEQ ID NO: 77 - protein, 233 aa, human
MSPSQLIGFLLLWVPASRGEIVLTQSPDFQSVTPKEKVTITCRASQSIGSSLHWYQQKPDQSPKLLIKYASQSFSGVPSRFSGSGSGTDFTLTINSLEAEDAAAYYCHQSSSLPLTFGGGTKVEIKRTVAAPSVFIFPPSDEQLKSGTASVVCLLNNFYPREAKVQWKVDNALQSGNSQESVTEQDSKDSTYSLSSTLTLSKADYEKHKVYACEVTHQGLSSPVTKSFNRGEC

SEQ ID NO: 78 - protein, 120 aa, human
QVQLVESGGGVVQPGRSLRLSCAASGFTFSNYGMHWVRQAPGKGLEWVAGIWNDGINKYHAHSVRGRFTISRDNSKNTLYLQMNSPRAEDTAVYYCARARSFDWLLFEFWGQGTLVTVSS

SEQ ID NO: 79 - protein, 109 aa, human
GEIVLTQSPATLSLSPGERATLSCRASQSVSSYLAWYQQKPGQAPRLLIYDASNRATGIPARFSGSGSGTDFTLTISSLEPEDFAVYYCQQRSNWPPLTFGGGTKVEIK

SEQ ID NO: 80 - protein, 120 aa, human
QVQLVESGGGVVQPGRSLRLSCAVSGFTFSNYGMHWVRQAPGKGLEWVAAIWNDGENKHHAGSVRGRFTISRDNSKNTLYLQMNSLRAEDTAVYYCARGRYFDWLLFEYWGQGTLVTVSS

SEQ ID NO: 81 - protein, 118 aa, human
EVQLMQSGAEVKKPGESLKISCKGSGYSFSFHWIAWVRQMPGKGLEWMGIIHPGASDTRYSPSFQGQVTISADNSNSATYLQWSSLKASDTAMYFCARQRELDYFDYWGQGTLVTVSS

SEQ ID NO: 82 - protein, 107 aa, human
EIVLTQSPDFQSVTPKEKVTITCRASQSIGSSLHWYQQKPDQSPKLLIKYASQSFSGVPSRFSGSGSGTDFTLTINSLEAEDAAAYYCHQSSSLPLTFGGGTKVEIK

SEQ ID NO: 83 - protein, 11 aa, human
RKCACVECPPC

SEQ ID NO: 84 - protein, 12 aa, human
RKCPPCVECPPC

SEQ ID NO: 85 - protein, 12 aa, human
RKANCCVECPPC

SEQ ID NO: 86 - protein, 12 aa, human
RKPNCCVECPPC